European Patent Application EP 4 273 307 A1, published November 8, 2023. Title: METHOD FOR RAPIDLY CONSTRUCTING CYCLIZED LIBRARY AND CYCLIZATION ADAPTERS. Applicant: MGI TECH CO., LTD. The sequence listing filed with the application follows.

SEQUENCE LISTING (4 sequences)

SEQ ID NO: 1 - DNA, 83 bp, Artificial Sequence
  Synthetic Construct
  misc_feature (32)..(41): n is a, c, g, or t
agtcggaggccaagcggtcttaggaagacaannnnnnnnnncaactccttggctcacagaacgacatggctacgatccgactt

SEQ ID NO: 2 - DNA, 41 bp, Artificial Sequence
  Synthetic Construct
agtcggatcgtagccatgtcgttctgtgagccaaggagttg

SEQ ID NO: 3 - DNA, 32 bp, Artificial Sequence
  Synthetic Construct
ttgtcttcctaagaccgcttggcctccgactt

SEQ ID NO: 4 - DNA, 93 bp, Artificial Sequence
  Synthetic Construct
  misc_feature (32)..(51): n is a, c, g, or t
agtcggaggccaagcggtcttaggaagacaannnnnnnnnnnnnnnnnnnncaactccttggctcacagaacgacatggctacgatccgactt